European Patent Application EP 4 710 945 A1, published March 18, 2026. Title: ANTI-EPIDERMAL GROWTH FACTOR RECEPTOR (EGFR) ANTIBODY-DRUG CONJUGATE AND USE THEREOF. Applicant: SHANGHAI HENLIUS BIOTECH, INC. The sequence listing filed with the application follows.

SEQUENCE LISTING (18 sequences)

SEQ ID NO: 1 - protein, 5 aa, synthetic construct
  source 1..5: note = MAB07 HC CDR1
NYGVH

SEQ ID NO: 2 - protein, 16 aa, synthetic construct
  source 1..16: note = MAB07 HC CDR2
VIWSGGNTDYGNEFTS

SEQ ID NO: 3 - protein, 11 aa, synthetic construct
  source 1..11: note = MAB07 HC CDR3
ALDYYDYEFAY

SEQ ID NO: 4 - protein, 11 aa, synthetic construct
  source 1..11: note = MAB07 LC CDR1
RASQSIGTNIH

SEQ ID NO: 5 - protein, 7 aa, synthetic construct
  source 1..7: note = MAB07 LC CDR2
YASESIS

SEQ ID NO: 6 - protein, 9 aa, synthetic construct
  source 1..9: note = MAB07 LC CDR3
QQNNNWPTS

SEQ ID NO: 7 - protein, 119 aa, synthetic construct
  source 1..119: note = MAB07 VH
EVQLVESGGGLVQPGGSLRLSCAASGFSLTNYGVHWVRQAPGKGLEWLGVIWSGGNTDYGNEFTSRFTISRDNAKNSLYLQMNSLRAEDTAVYYCARALDYYDYEFAYWGQGTMVTVSS

SEQ ID NO: 8 - protein, 110 aa, synthetic construct
  source 1..110: note = MAB07 VL
EIVLTQSPATLSLSPGERATLSCRASQSIGTNIHWYQQKPGQAPRLLIKYASESISGIPARFSGSGSGTDFTLTISSLEPEDFAVYYCQQNNNWPTSFGGGTKVEIKRTV

SEQ ID NO: 9 - protein, 449 aa, synthetic construct
  source 1..449: note = MAB07 HC
EVQLVESGGGLVQPGGSLRLSCAASGFSLTNYGVHWVRQAPGKGLEWLGVIWSGGNTDYGNEFTSRFTISRDNAKNSLYLQMNSLRAEDTAVYYCARALDYYDYEFAYWGQGTMVTVSSASTKGPSVFPLAPSSKSTSGGTAALGCLVKDYFPEPVTVSWNSGALTSGVHTFPAVLQSSGLYSLSSVVTVPSSSLGTQTYICNVNHKPSNTKVDKRVEPKSCDKTHTCPPCPAPELLGGPSVFLFPPKPKDTLMISRTPEVTCVVVDVSHEDPEVKFNWYVDGVEVHNAKTKPREEQYNSTYRVVSVLTVLHQDWLNGKEYKCKVSNKALPAPIEKTISKAKGQPREPQVYTLPPSREEMTKNQVSLTCLVKGFYPSDIAVEWESNGQPENNYKTTPPVLDSDGSFFLYSKLTVDKSRWQQGNVFSCSVMHEALHNHYTQKSLSLSPGK

SEQ ID NO: 10 - protein, 214 aa, synthetic construct
  source 1..214: note = MAB07 LC
EIVLTQSPATLSLSPGERATLSCRASQSIGTNIHWYQQKPGQAPRLLIKYASESISGIPARFSGSGSGTDFTLTISSLEPEDFAVYYCQQNNNWPTSFGGGTKVEIKRTVAAPSVFIFPPSDEQLKSGTASVVCLLNNFYPREAKVQWKVDNALQSGNSQESVTEQDSKDSTYSLSSTLTLSKADYEKHKVYACEVTHQGLSSPVTKSFNRGEC

SEQ ID NO: 11 - protein, 449 aa, synthetic construct
  source 1..449: note = Cetuximab HC
QVQLKQSGPGLVQPSQSLSITCTVSGFSLTNYGVHWVRQSPGKGLEWLGVIWSGGNTDYNTPFTSRLSINKDNSKSQVFFKMNSLQSNDTAIYYCARALTYYDYEFAYWGQGTLVTVSAASTKGPSVFPLAPSSKSTSGGTAALGCLVKDYFPEPVTVSWNSGALTSGVHTFPAVLQSSGLYSLSSVVTVPSSSLGTQTYICNVNHKPSNTKVDKRVEPKSCDKTHTCPPCPAPELLGGPSVFLFPPKPKDTLMISRTPEVTCVVVDVSHEDPEVKFNWYVDGVEVHNAKTKPREEQYNSTYRVVSVLTVLHQDWLNGKEYKCKVSNKALPAPIEKTISKAKGQPREPQVYTLPPSREEMTKNQVSLTCLVKGFYPSDIAVEWESNGQPENNYKTTPPVLDSDGSFFLYSKLTVDKSRWQQGNVFSCSVMHEALHNHYTQKSLSLSPGK

SEQ ID NO: 12 - protein, 214 aa, synthetic construct
  source 1..214: note = Cetuximab LC
DILLTQSPVILSVSPGERVSFSCRASQSIGTNIHWYQQRTNGSPRLLIKYASESISGIPSRFSGSGSGTDFTLSINSVESEDIADYYCQQNNNWPTTFGAGTKLELKRTVAAPSVFIFPPSDEQLKSGTASVVCLLNNFYPREAKVQWKVDNALQSGNSQESVTEQDSKDSTYSLSSTLTLSKADYEKHKVYACEVTHQGLSSPVTKSFNRGEC

SEQ ID NO: 13 - protein, 621 aa, synthetic construct [sequence omitted]

SEQ ID NO: 14 - protein, 621 aa, synthetic construct
  source 1..621: note = Cynomolgus EGFR ECD
LEEKKVCQGTSNKLTQLGTFEDHFLSLQRMFNNCEVVLGNLEITYVQRNYDLSFLKTIQEVAGYVLIALNTVERIPLENLQIIRGNMYYENSYALAVLSNYDANKTGLKELPMRNLQEILHGAVRFSNNPALCNVESIQWRDIVSSEFLSNMSMDFQNHLGSCQKCDPSCPNGSCWGAGEENCQKLTKIICAQQCSGRCRGKSPSDCCHNQCAAGCTGPRESDCLVCRKFRDEATCKDTCPPLMLYNPTTYQMDVNPEGKYSFGATCVKKCPRNYVVTDHGSCVRACGADSYEMEEDGVRKCKKCEGPCRKVCNGIGIGEFKDTLSINATNIKHFKNCTSISGDLHILPVAFRGDSFTHTPPLDPQELDILKTVKEITGFLLIQAWPENRTDLHAFENLEIIRGRTKQHGQFSLAVVSLNITSLGLRSLKEISDGDVIISGNKNLCYANTINWKKLFGTSSQKTKIISNRGENSCKATGQVCHALCSPEGCWGPEPRDCVSCQNVSRGRECVDKCNVLEGEPREFVENSECIQCHPECLPQVMNITCTGRGPDNCIQCAHYIDGPHCVKTCPAGVMGENNTLVWKYADAGHVCHLCHPNCTYGCTGPGLEGCARNGPKIPS

SEQ ID NO: 15 - protein, 622 aa, synthetic construct
  source 1..622: note = Rat EGFR ECD
LEEKKVCQGTSNRLTQLGTFEDHFLSLQRMFNNCEVVLGNLEITYVQRNYDLSFLKTIQEVAGYVLIALNTVERIPLENLQIIRGNALYENTYALAVLSNYGTNKTGLRELPMRNLQEILIGAVRFSNNPILCNMETIQWRDIVQDVFLSNMSMDVQRHLTGCPKCDPSCPNGSCWGRGEENCQKLTKIICAQQCSRRCRGRSPSDCCHNQCAAGCTGPRESDCLVCHRFRDEATCKDTCPPLMLYNPTTYQMDVNPEGKYSFGATCVKKCPRNYVVTDHGSCVRACGPDYYEVEEDGVSKCKKCDGPCRKVCNGIGIGEFKDTLSINATNIKHFKYCTAISGDLHILPVAFKGDSFTRTPPLDPRELEILKTVKEITGFLLIQAWPENWTDLHAFENLEIIRGRTKQHGQFSLAVVGLNITSLGLRSLKEISDGDVIISGNRNLCYANTINWKKLFGTPNQKTKIMNNRAEKDCKATNHVCNPLCSSEGCWGPEPTDCVSCQNVSRGRECVDKCNILEGEPREFVENSECIQCHPECLPQTMNITCTGRGPDNCIKCAHYVDGPHCVKTCPSGIMGENNTLVWKFADANNVCHLCHANCTYGCAGPGLKGCQQPEGPKIPS

SEQ ID NO: 16 - protein, 623 aa, synthetic construct
  source 1..623: note = Mice EGFR ECD
LEEKKVCQGTSNRLTQLGTFEDHFLSLQRMYNNCEVVLGNLEITYVQRNYDLSFLKTIQEVAGYVLIALNTVERIPLENLQIIRGNALYENTYALAILSNYGTNRTGLRELPMRNLQEILIGAVRFSNNPILCNMDTIQWRDIVQNVFMSNMSMDLQSHPSSCPKCDPSCPNGSCWGGGEENCQKLTKIICAQQCSHRCRGRSPSDCCHNQCAAGCTGPRESDCLVCQKFQDEATCKDTCPPLMLYNPTTYQMDVNPEGKYSFGATCVKKCPRNYVVTDHGSCVRACGPDYYEVEEDGIRKCKKCDGPCRKVCNGIGIGEFKDTLSINATNIKHFKYCTAISGDLHILPVAFKGDSFTRTPPLDPRELEILKTVKEITGFLLIQAWPDNWTDLHAFENLEIIRGRTKQHGQFSLAVVGLNITSLGLRSLKEISDGDVIISGNRNLCYANTINWKKLFGTPNQKTKIMNNRAEKDCKAVNHVCNPLCSSEGCWGPEPRDCVSCQNVSRGRECVEKCNILEGEPREFVENSECIQCHPECLPQAMNITCTGRGPDNCIQCAHYIDGPHCVKTCPAGIMGENNTLVWKYADANNVCHLCHANCTYGCAGPGLQGCEVWPSGPKIPS

SEQ ID NO: 17 - protein, 443 aa, synthetic construct
  source 1..443: note = Serplulimab HC
QVQLVESGGGLVKPGGSLRLSCAASGFTFSNYGMSWIRQAPGKGLEWVSTISGGGSNIYYADSVKGRFTISRDNAKNSLYLQMNSLRAEDTAVYYCVSYYYGIDFWGQGTSVTVSSASTKGPSVFPLAPCSRSTSESTAALGCLVKDYFPEPVTVSWNSGALTSGVHTFPAVLQSSGLYSLSSVVTVPSSSLGTKTYTCNVDHKPSNTKVDKRVESKYGPPCPPCPAPEFLGGPSVFLFPPKPKDTLMISRTPEVTCVVVDVSQEDPEVQFNWYVDGVEVHNAKTKPREEQFNSTYRVVSVLTVLHQDWLNGKEYKCKVSNKGLPSSIEKTISKAKGQPREPQVYTLPPSQEEMTKNQVSLTCLVKGFYPSDIAVEWESNGQPENNYKTTPPVLDSDGSFFLYSRLTVDKSRWQEGNVFSCSVMHEALHNHYTQKSLSLSLGK

SEQ ID NO: 18 - protein, 214 aa, synthetic construct
  source 1..214: note = Serplulimab LC
DIQMTQSPSSLSASVGDRVTITCKASQDVTTAVAWYQQKPGKAPKLLIYWASTRHTGVPSRFSGSGSGTDFTLTISSLQPEDFATYYCQQHYTIPWTFGGGTKLEIKRTVAAPSVFIFPPSDEQLKSGTASVVCLLNNFYPREAKVQWKVDNALQSGNSQESVTEQDSKDSTYSLSSTLTLSKADYEKHKVYACEVTHQGLSSPVTKSFNRGEC